European Patent Specification EP 4 463 465 B1, published January 7, 2026. Title: HIGH AFFINITY PURIFICATION OF FERRITIN. Applicant: Navigo Proteins GmbH. Application EP. The sequence listing filed with the application follows.

SEQUENCE LISTING (12 sequences)

SEQ ID NO: 1 - protein, 56 aa, synthetic construct
  REGION 1..56: note = ferritin binding protein
  REGION 5..6: note = misc_feature - X can be any naturally occurring amino acid
  SITE 8: note = misc_feature - X can be any naturally occurring amino acid
  REGION 12..13: note = misc_feature - X can be any naturally occurring amino acid
  SITE 16: note = misc_feature - X can be any naturally occurring amino acid
  SITE 18: note = misc_feature - X can be any naturally occurring amino acid
  SITE 41: note = misc_feature - X can be any naturally occurring amino acid
  SITE 44: note = misc_feature - X can be any naturally occurring amino acid
  SITE 48: note = misc_feature - X can be any naturally occurring amino acid
  SITE 52: note = misc_feature - X can be any naturally occurring amino acid
AKFDXXQXYADXXILXLXNLTEEQRNAFRQSLSDDPSVSWXVLXEARXLNEXQAPK

SEQ ID NO: 2 - protein, 56 aa, synthetic construct
  REGION 1..56: note = ferritin binding protein (218990)
AKFDQWQSYADHQILKLPNLTEEQRNAFRQSLSDDPSVSWEVLWEARELNESQAPK

SEQ ID NO: 3 - protein, 56 aa, synthetic construct
  REGION 1..56: note = ferritin binding protein (218989)
AKFDAYQSYADKEILQLPNLTEEQRNAFRQSLSDDPSVSWEVLQEARVLNESQAPK

SEQ ID NO: 4 - protein, 56 aa, synthetic construct
  REGION 1..56: note = ferritin binding protein (218894)
AKFDQFQLYADKEILELFNLTEEQRNAFRQSLSDDPSVSWYVLWEARMLNEAQAPK

SEQ ID NO: 5 - protein, 173 aa, synthetic construct
  REGION 1..173: note = fusion protein comprising SEQ ID NO: 2 (219126)
AKFDQWQSYADHQILKLPNLTEEQRNAFRQSLSDDPSVSWEVLWEARELNESQAPKIAAQHDKIQQAADKEILHLPNLTEEQRNKFRQSLRDDPSVSAEILAEAKKLNDAQAPKIAAQHDKIQQAADKEILHLPNLTEEQRNKFRQSLRDDPSVSAEILAEAKKLNDAQAPKC

SEQ ID NO: 6 - protein, 231 aa, synthetic construct
  REGION 1..231: note = fusion protein comprising SEQ ID NO: 2 (dimer)(219127)
AKFDQWQSYADHQILKLPNLTEEQRNAFRQSLSDDPSVSWEVLWEARELNESQAPKIAAKFDQWQSYADHQILKLPNLTEEQRNAFRQSLSDDPSVSWEVLWEARELNESQAPKIAAQHDKIQQAADKEILHLPNLTEEQRNKFRQSLRDDPSVSAEILAEAKKLNDAQAPKIAAQHDKIQQAADKEILHLPNLTEEQRNKFRQSLRDDPSVSAEILAEAKKLNDAQAPKC

SEQ ID NO: 7 - protein, 173 aa, synthetic construct
  REGION 1..173: note = fusion protein comprising SEQ ID NO: 3 (219124)
AKFDAYQSYADKEILQLPNLTEEQRNAFRQSLSDDPSVSWEVLQEARVLNESQAPKIAAQHDKIQQAADKEILHLPNLTEEQRNKFRQSLRDDPSVSAEILAEAKKLNDAQAPKIAAQHDKIQQAADKEILHLPNLTEEQRNKFRQSLRDDPSVSAEILAEAKKLNDAQAPKC

SEQ ID NO: 8 - protein, 231 aa, synthetic construct
  REGION 1..231: note = fusion protein comprising SEQ ID NO: 3 (dimer)(219125)
AKFDAYQSYADKEILQLPNLTEEQRNAFRQSLSDDPSVSWEVLQEARVLNESQAPKIAAKFDAYQSYADKEILQLPNLTEEQRNAFRQSLSDDPSVSWEVLQEARVLNESQAPKIAAQHDKIQQAADKEILHLPNLTEEQRNKFRQSLRDDPSVSAEILAEAKKLNDAQAPKIAAQHDKIQQAADKEILHLPNLTEEQRNKFRQSLRDDPSVSAEILAEAKKLNDAQAPKC

SEQ ID NO: 9 - protein, 173 aa, synthetic construct
  REGION 1..173: note = fusion protein comprising SEQ ID NO: 4 (219122)
AKFDQFQLYADKEILELFNLTEEQRNAFRQSLSDDPSVSWYVLWEARMLNEAQAPKIAAQHDKIQQAADKEILHLPNLTEEQRNKFRQSLRDDPSVSAEILAEAKKLNDAQAPKIAAQHDKIQQAADKEILHLPNLTEEQRNKFRQSLRDDPSVSAEILAEAKKLNDAQAPKC

SEQ ID NO: 10 - protein, 231 aa, synthetic construct
  REGION 1..231: note = fusion protein comprising SEQ ID NO: 4 (dimer)(219123)
AKFDQFQLYADKEILELFNLTEEQRNAFRQSLSDDPSVSWYVLWEARMLNEAQAPKIAAKFDQFQLYADKEILELFNLTEEQRNAFRQSLSDDPSVSWYVLWEARMLNEAQAPKIAAQHDKIQQAADKEILHLPNLTEEQRNKFRQSLRDDPSVSAEILAEAKKLNDAQAPKIAAQHDKIQQAADKEILHLPNLTEEQRNKFRQSLRDDPSVSAEILAEAKKLNDAQAPKC

SEQ ID NO: 11 - protein, 56 aa, synthetic construct
  REGION 1..56: note = non ferritin binding protein
AQHDKIQQAADKEILHLPNLTEEQRNKFRQSLRDDPSVSAEILAEAKKLNDAQAPK

SEQ ID NO: 12 - protein, 165 aa, Homo sapiens [sequence omitted]